European Patent Application EP 4 512 420 A1, published February 26, 2025. Title: Composition for reducing the size or volume of the target tissue or a kit comprising thereof. Applicant: 에스케이바이오사이언스(주). The sequence listing filed with the application follows.

SEQUENCE LISTING (21 sequences)

SEQ ID NO: 1 - DNA, 2334 bp, Yellow fever virus
  source 1..2334: mol_type = other DNA
atgtctggtcgtaaagctcagggaaaaaccctgggcgtcaatatggtacgacgaggagttcgctccttgtcaaacaaaataaaacaaaaaacaaaacaaattggaaacagacctggaccttcaagaggtgttcaaggatttatctttttctttttgttcaacattttgactggaaaaaagatcacagcccacctaaagaggttgtggaaaatgctggacccaagacaaggcttggctgttctaaggaaagtcaagagagtggtggccagtttgatgagaggattgtcctcaaggaaacgccgttcccatgatgttctgactgtgcaattcctaattttgggaatgctgttgatgacgggtggagtgaccttggtgcggaaaaacagatggttgctcctaaatgtgacatctgaggacctcgggaaaacattctctgtgggcacaggcaactgcacaacaaacattttggaagccaagtactggtgcccagactcaatggaatacaactgtcccaatctcagtccaagagaggagccagatgacattgattgctggtgctatggggtggaaaacgttagagtcgcatatggtaagtgtgactcagcaggcaggtctaggaggtcaagaagggccattgacttgcctacgcatgaaaaccatggtttgaagacccggcaagaaaaatggatgactggaagaatgggtgaaaggcaactccaaaagattgagagatggttcgtgaggaaccccttttttgcagtgacggctctgaccattgcctaccttgtgggaagcaacatgacgcaacgagtcgtgattgccctactggtcttggctgttggtccggcctactcagctcactgcattggaattactgacagggatttcattgagggggtgcatggaggaacttgggtttcagctaccctggagcaagacaagtgtgtcactgttatggcccctgacaagccttcattggacatctcactagagacagtagccattgatagacctgctgaggtgaggaaagtgtgttacaatgcagttctcactcatgtgaagattaatgacaagtgccccagcactggagaggcccacctagctgaagagaacgaaggggacaatgcgtgcaagcgcacttattctgatagaggctggggcaatggctgtggcctatttgggaaagggagcattgtggcatgcgccaaattcacttgtgccaaatccatgagtttgtttgaggttgatcagaccaaaattcagtatgtcatcagagcacaattgcatgtaggggccaagcaggaaaattggaataccgacattaagactctcaagtttgatgccctgtcaggctcccaggaagtcgagttcattgggtatggaaaagctacactggaatgccaggtgcaaactgcggtggactttggtaacagttacatcgctgagatggaaacagagagctggatagtggacagacagtgggcccaggacttgaccctgccatggcagagtggaagtggcggggtgtggagagagatgcatcatcttgtcgaatttgaacctccgcatgccgccactatcagagtactggccctgggaaaccaggaaggctccttgaaaacagctcttactggcgcaatgagggttacaaaggacacaaatgacaacaacctttacaaactacatggtggacatgtttcttgcagagtgaaattgtcagctttgacactcaaggggacatcctacaaaatatgcactgacaaaatgttttttgtcaagaacccaactgacactggccatggcactgttgtgatgcaggtgaaagtgtcaaaaggagccccctgcaggattccagtgatagtagctgatgatcttacagcggcaatcaataaaggcattttggttacagttaaccccatcgcctcaaccaatgatgatgaagtgctgattgaggtgaacccaccttttggagacagctacattatcgttgggagaggagattcacgtctcacttaccagtggcacaaagagggaagctcaataggaaagttgttcactcagaccatgaaaggcgtggaacgcctggccgtcatgggagacaccgcctgggatttcagctccgctggagggttcttcacttcggttgggaaaggaattcatacggtgtttggctctgcctttcaggggctatttggcggcttgaactggataacaaaggtcatcatgggggcggtacttatatgggttggcatcaacacaagaaacatgacaatgtccatgagcatgatcttggtaggagtgatcatgatgtttttgtctctaggagttggggcg

SEQ ID NO: 2 - RNA, 2617 nt, Yellow fever virus
  source 1..2617: mol_type = mRNA
gagagcagcgctgggtgttcaggggccaaggccaccatgtctggtcgtaaagctcagggaaaaaccctgggcgtcaatatggtacgacgaggagttcgctccttgtcaaacaaaataaaacaaaaaacaaaacaaattggaaacagacctggaccttcaagaggtgttcaaggatttatctttttctttttgttcaacattttgactggaaaaaagatcacagcccacctaaagaggttgtggaaaatgctggacccaagacaaggcttggctgttctaaggaaagtcaagagagtggtggccagtttgatgagaggattgtcctcaaggaaacgccgttcccatgatgttctgactgtgcaattcctaattttgggaatgctgttgatgacgggtggagtgaccttggtgcggaaaaacagatggttgctcctaaatgtgacatctgaggacctcgggaaaacattctctgtgggcacaggcaactgcacaacaaacattttggaagccaagtactggtgcccagactcaatggaatacaactgtcccaatctcagtccaagagaggagccagatgacattgattgctggtgctatggggtggaaaacgttagagtcgcatatggtaagtgtgactcagcaggcaggtctaggaggtcaagaagggccattgacttgcctacgcatgaaaaccatggtttgaagacccggcaagaaaaatggatgactggaagaatgggtgaaaggcaactccaaaagattgagagatggttcgtgaggaaccccttttttgcagtgacggctctgaccattgcctaccttgtgggaagcaacatgacgcaacgagtcgtgattgccctactggtcttggctgttggtccggcctactcagctcactgcattggaattactgacagggatttcattgagggggtgcatggaggaacttgggtttcagctaccctggagcaagacaagtgtgtcactgttatggcccctgacaagccttcattggacatctcactagagacagtagccattgatagacctgctgaggtgaggaaagtgtgttacaatgcagttctcactcatgtgaagattaatgacaagtgccccagcactggagaggcccacctagctgaagagaacgaaggggacaatgcgtgcaagcgcacttattctgatagaggctggggcaatggctgtggcctatttgggaaagggagcattgtggcatgcgccaaattcacttgtgccaaatccatgagtttgtttgaggttgatcagaccaaaattcagtatgtcatcagagcacaattgcatgtaggggccaagcaggaaaattggaataccgacattaagactctcaagtttgatgccctgtcaggctcccaggaagtcgagttcattgggtatggaaaagctacactggaatgccaggtgcaaactgcggtggactttggtaacagttacatcgctgagatggaaacagagagctggatagtggacagacagtgggcccaggacttgaccctgccatggcagagtggaagtggcggggtgtggagagagatgcatcatcttgtcgaatttgaacctccgcatgccgccactatcagagtactggccctgggaaaccaggaaggctccttgaaaacagctcttactggcgcaatgagggttacaaaggacacaaatgacaacaacctttacaaactacatggtggacatgtttcttgcagagtgaaattgtcagctttgacactcaaggggacatcctacaaaatatgcactgacaaaatgttttttgtcaagaacccaactgacactggccatggcactgttgtgatgcaggtgaaagtgtcaaaaggagccccctgcaggattccagtgatagtagctgatgatcttacagcggcaatcaataaaggcattttggttacagttaaccccatcgcctcaaccaatgatgatgaagtgctgattgaggtgaacccaccttttggagacagctacattatcgttgggagaggagattcacgtctcacttaccagtggcacaaagagggaagctcaataggaaagttgttcactcagaccatgaaaggcgtggaacgcctggccgtcatgggagacaccgcctgggatttcagctccgctggagggttcttcacttcggttgggaaaggaattcatacggtgtttggctctgcctttcaggggctatttggcggcttgaactggataacaaaggtcatcatgggggcggtacttatatgggttggcatcaacacaagaaacatgacaatgtccatgagcatgatcttggtaggagtgatcatgatgtttttgtctctaggagttggggcgtgagctggagcctcggtggccatgcttcttgccccttgggcctccccccagcccctcctccccttcctgcacccgtacccccgtggtctttgaataaagtctgagtgggcggcaaaaaaaaaaaaaaaaaaaaaaaaaaaaaaagcatatgactaaaaaaaaaaaaaaaaaaaaaaaaaaaaaaaaaaaaaaaaaaaaaaaaaaaaaaaaaaaaaaaaaaaaaaaaaaagagacgccgctgatcagc

SEQ ID NO: 3 - DNA, 1872 bp, varicella-zoster virus
  source 1..1872: mol_type = genomic DNA
atgggaaccgtgaacaagcctgtggtcggcgtgctgatgggctttggcattatcacaggcaccctgcggatcaccaaccctgtgcgggccagcgttctgagatacgacgacttccacatcgacgaggacaagctggacaccaacagcgtctacgagccctattaccattctgatcacgccgaatcttcttgggtgaatagaggcgagtctagcagaaaggcctatgaccacaactccccatacatttggcctcgtaacgactacgacggcttcctggaaaacgcccacgagcaccacggcgtgtacaaccagggaagaggcatcgacagcggagagagactgatgcagccaacccagatgagcgcccaggaggacctgggagacgacaccggcatccacgttatccccacactgaacggcgacgatagacacaagatcgtgaacgtggatcagagacagtacggcgatgtgttcaagggcgacctgaatcctaaacctcagggccaaagactgatcgaggtgtccgtggaagaaaatcaccccttcaccctgcgggcccctatccagcggatctacggcgtgcggtacacagagacatggtccttcctgccatctctgacctgcaccggggacgccgctcctgccatccaacacatctgtctgaagcacaccacctgcttccaggatgtggtcgtggacgtggattgcgccgaaaacacaaaagaagatcagctggccgagatcagctacagattccaagggaagaaggaggccgaccagccctggatcgtggtgaacaccagcacactgttcgacgagctggaactggaccctcctgagatcgagcctggcgtgctgaaagtgctgaggaccgagaaacagtacctgggcgtgtacatctggaatatgagaggcagcgacggcacctccacctacgccacatttctggtcacctggaagggcgatgagaagacccgcaaccccacccctgcagtgacccctcaacctagaggcgccgagttccacatgtggaactaccactctcatgtgttcagcgtgggcgacacgttctctctggctatgcacctgcagtataagatccacgaggctccttttgatctgctgctggaatggctgtacgtgcccatcgaccctacctgtcagcctatgcggctgtatagcacatgtctgtaccaccctaacgcccctcagtgcctgagccacatgaacagcggatgtacctttaccagcccgcacctggcccagagagtggccagcaccgtgtaccagaattgcgagcacgccgataactacaccgcctactgcctgggaattagccacatggaacccagctttggcctgatcctgcacgacggcggcacaacccttaaattcgtggacacacctgagagtctgagcggactgtacgtgttcgtggtgtacttcaacggccacgtggaagccgtggcctacaccgtggtctccaccgtggatcatttcgttaatgccatcgaggaacggggcttcccccccacagctggccagccacctgctacaacaaagcccaaggaaatcacacctgtgaaccccggcacaagcccactgctcagatacgccgcatggaccggcggcctggccgccgtggtgctgctatgcctggtgatcttcctgatctgcaccgccaagagaatgagagtgaaggcctaccgggtggacaaaagcccctacaaccagagcatgtactacgccggcctccctgttgacgacttcgaggacagcgagtccactgatacagaggaagaatttggcaacgccatcggcggtagccacggaggaagcagctacaccgtgtacatcgacaagaccagatga

SEQ ID NO: 4 - RNA, 2152 nt, varicella-zoster virus
  source 1..2152: mol_type = mRNA
gagagcagcgctgggtgttcaggggccaaggccaccatgggaaccgtgaacaagcctgtggtcggcgtgctgatgggctttggcattatcacaggcaccctgcggatcaccaaccctgtgcgggccagcgttctgagatacgacgacttccacatcgacgaggacaagctggacaccaacagcgtctacgagccctattaccattctgatcacgccgaatcttcttgggtgaatagaggcgagtctagcagaaaggcctatgaccacaactccccatacatttggcctcgtaacgactacgacggcttcctggaaaacgcccacgagcaccacggcgtgtacaaccagggaagaggcatcgacagcggagagagactgatgcagccaacccagatgagcgcccaggaggacctgggagacgacaccggcatccacgttatccccacactgaacggcgacgatagacacaagatcgtgaacgtggatcagagacagtacggcgatgtgttcaagggcgacctgaatcctaaacctcagggccaaagactgatcgaggtgtccgtggaagaaaatcaccccttcaccctgcgggcccctatccagcggatctacggcgtgcggtacacagagacatggtccttcctgccatctctgacctgcaccggggacgccgctcctgccatccaacacatctgtctgaagcacaccacctgcttccaggatgtggtcgtggacgtggattgcgccgaaaacacaaaagaagatcagctggccgagatcagctacagattccaagggaagaaggaggccgaccagccctggatcgtggtgaacaccagcacactgttcgacgagctggaactggaccctcctgagatcgagcctggcgtgctgaaagtgctgaggaccgagaaacagtacctgggcgtgtacatctggaatatgagaggcagcgacggcacctccacctacgccacatttctggtcacctggaagggcgatgagaagacccgcaaccccacccctgcagtgacccctcaacctagaggcgccgagttccacatgtggaactaccactctcatgtgttcagcgtgggcgacacgttctctctggctatgcacctgcagtataagatccacgaggctccttttgatctgctgctggaatggctgtacgtgcccatcgaccctacctgtcagcctatgcggctgtatagcacatgtctgtaccaccctaacgcccctcagtgcctgagccacatgaacagcggatgtacctttaccagcccgcacctggcccagagagtggccagcaccgtgtaccagaattgcgagcacgccgataactacaccgcctactgcctgggaattagccacatggaacccagctttggcctgatcctgcacgacggcggcacaacccttaaattcgtggacacacctgagagtctgagcggactgtacgtgttcgtggtgtacttcaacggccacgtggaagccgtggcctacaccgtggtctccaccgtggatcatttcgttaatgccatcgaggaacggggcttcccccccacagctggccagccacctgctacaacaaagcccaaggaaatcacacctgtgaaccccggcacaagcccactgctcagatacgccgcatggaccggcggcctggccgccgtggtgctgctatgcctggtgatcttcctgatctgcaccgccaagagaatgagagtgaaggcctaccgggtggacaaaagcccctacaaccagagcatgtactacgccggcctccctgttgacgacttcgaggacagcgagtccactgatacagaggaagaatttggcaacgccatcggcggtagccacggaggaagcagctacaccgtgtacatcgacaagaccagatgagctggagcctcggtggccatgcttcttgccccttgggcctccccccagcccctcctccccttcctgcacccgtacccccgtggtctttgaataaagtctgagtgggcggcaaaaaaaaaaaaaaaaaaaaaaaaaaaaaaagcatatgactaaaaaaaaaaaaaaaaaaaaaaaaaaaaaaaaaaaaaaaaaaaaaaaaaaaaaaaaaaaaaaaaaaaaaaaaaaagagacgccgctgatcagc

SEQ ID NO: 5 - DNA, 2358 bp, Rubella virus
  source 1..2358: mol_type = genomic DNA
ggcgctccccaggccttcctggccggcctgctgctggctgctgtggccgtgggcacagctagagccggcctccaacctagagccgacatggccgccccacccacactgcctcagccccctcgggcccacggccaacactacggccaccaccaccatcagctgccattcctgggccacgatggccaccacggcggcacactgagggtgggccagcaccacagaaacgccagcgacgtgctgcctgggcactggctgcagggaggctggggatgttacaacctgagcgactggcaccagggcacccacgtgtgccacaccaagcacatggacttctggtgcgtggaacacgacagaccccctcctgccacccccacaccactgacaaccgctgctaactctaccaccgccgccacacctgccaccgccccagctccatgtcacgccggcctgaacgacagctgtggcggctttctcagcggctgtggccctatgcggctgcggcacggcgctgacacccggtgcggcagactgatttgcggcctgtccaccacagcccaatacccccccaccagattcggctgcgccatgagatggggcctgcctccttgggagctggtggtgctgaccgcccggcctgaggacggctggacctgcagaggagtgccggcccacccaggcaccagatgtccagaactggtgtcccctatgggaagagccacctgttctcctgcttcagccctgtggctggctaccgccaacgccctgagcctggaccacgccctggccgcttttgtgctgctggtcccttgggtcctgatcttcatggtgtgcagaagaacatgtagaagacggggcgccgccgcggctctgacagccgtggtgctgcagggctacaaccccccagcctacggcgaggaagccttcacctacctctgcaccgcccctggctgcgccacccaagcccctgtgcctgtcagactggcaggcgtgcggtttgagagcaagatcgtggacggcggctgcttcgccccttgggacttggaggccaccggcgcctgcatctgcgaaatccctacagatgtgtcctgcgagggcctgggcgcttgggtgcccaccgcaccctgcgccagaatctggaacggaactcagcgagcctgcacattctgggctgtgaatgcctacagcagcggcggatacgcccagctggccagctacttcaaccctggcggttcttattacaagcagtaccaccctaccgcctgcgaggtggaacctgccttcggccattctgacgccgcctgctggggattccccacagatacagtgatgtctgtgttcgccctggccagctacgtgcagcacccacacaaaaccgtgagagttaagtttcacaccgagacaagaacagtctggcagctgagcgtggccggagtgtcttgtaacgtgacaacagagcatcccttctgcaacacccctcacggccagttagaggtgcaagtgcctcctgatcctggcgacctggtggagtacatcatgaaccacacaggcaaccagcagtccagatggggcctgggaagccccaactgccacggccctgattgggccagccctgtgtgtcagagacactctcctgactgcagccggctggtgggcgctacccctgaaagacctagactgcgcctggtggatgccgacgaccccctgctcagaaccgctcctggccccggcgaggtgtgggtcacacctgtgatcggcagccaggcccggaagtgcgggctgcacatcagagccggcccttacggccacgccaccgtcgaaatgcctgagtggattcacgcccacaccacaagcgacccctggcacccccccggccccctgggcttgaagttcaagaccgtgcggcccgtggccctgcctaggaccctggcccctcctcggaatgtgcgggtgaccggctgttaccagtgcggtactcccgctctggtggagggcctcgcccctggcggaggcaattgtcacctgaccgtcaacggagaggacctgggcgcctttcctcctggcaagttcgtgaccgccgccctgctgaataccccccctccttatcaggtgtcctgcggcggggaaagcgatagagccagcgcccgcgtcatcgaccctgccgcccagagcttcaccggagttgtgtacggaacccacacaaccgcagttagtgaaacaagacagacctgggccgagtgggcggctgcccattggtggcagctgaccctgggcgctatctgcgccctgctgctcgctggactgcttgcctgttgtgccaaatgcctgtactacctgcggggtgccatcgccccaagatga

SEQ ID NO: 6 - RNA, 2641 nt, Rubella virus
  source 1..2641: mol_type = mRNA
gagagcagcgctgggtgttcaggggccaaggccaccatgggcgctccccaggccttcctggccggcctgctgctggctgctgtggccgtgggcacagctagagccggcctccaacctagagccgacatggccgccccacccacactgcctcagccccctcgggcccacggccaacactacggccaccaccaccatcagctgccattcctgggccacgatggccaccacggcggcacactgagggtgggccagcaccacagaaacgccagcgacgtgctgcctgggcactggctgcagggaggctggggatgttacaacctgagcgactggcaccagggcacccacgtgtgccacaccaagcacatggacttctggtgcgtggaacacgacagaccccctcctgccacccccacaccactgacaaccgctgctaactctaccaccgccgccacacctgccaccgccccagctccatgtcacgccggcctgaacgacagctgtggcggctttctcagcggctgtggccctatgcggctgcggcacggcgctgacacccggtgcggcagactgatttgcggcctgtccaccacagcccaatacccccccaccagattcggctgcgccatgagatggggcctgcctccttgggagctggtggtgctgaccgcccggcctgaggacggctggacctgcagaggagtgccggcccacccaggcaccagatgtccagaactggtgtcccctatgggaagagccacctgttctcctgcttcagccctgtggctggctaccgccaacgccctgagcctggaccacgccctggccgcttttgtgctgctggtcccttgggtcctgatcttcatggtgtgcagaagaacatgtagaagacggggcgccgccgcggctctgacagccgtggtgctgcagggctacaaccccccagcctacggcgaggaagccttcacctacctctgcaccgcccctggctgcgccacccaagcccctgtgcctgtcagactggcaggcgtgcggtttgagagcaagatcgtggacggcggctgcttcgccccttgggacttggaggccaccggcgcctgcatctgcgaaatccctacagatgtgtcctgcgagggcctgggcgcttgggtgcccaccgcaccctgcgccagaatctggaacggaactcagcgagcctgcacattctgggctgtgaatgcctacagcagcggcggatacgcccagctggccagctacttcaaccctggcggttcttattacaagcagtaccaccctaccgcctgcgaggtggaacctgccttcggccattctgacgccgcctgctggggattccccacagatacagtgatgtctgtgttcgccctggccagctacgtgcagcacccacacaaaaccgtgagagttaagtttcacaccgagacaagaacagtctggcagctgagcgtggccggagtgtcttgtaacgtgacaacagagcatcccttctgcaacacccctcacggccagttagaggtgcaagtgcctcctgatcctggcgacctggtggagtacatcatgaaccacacaggcaaccagcagtccagatggggcctgggaagccccaactgccacggccctgattgggccagccctgtgtgtcagagacactctcctgactgcagccggctggtgggcgctacccctgaaagacctagactgcgcctggtggatgccgacgaccccctgctcagaaccgctcctggccccggcgaggtgtgggtcacacctgtgatcggcagccaggcccggaagtgcgggctgcacatcagagccggcccttacggccacgccaccgtcgaaatgcctgagtggattcacgcccacaccacaagcgacccctggcacccccccggccccctgggcttgaagttcaagaccgtgcggcccgtggccctgcctaggaccctggcccctcctcggaatgtgcgggtgaccggctgttaccagtgcggtactcccgctctggtggagggcctcgcccctggcggaggcaattgtcacctgaccgtcaacggagaggacctgggcgcctttcctcctggcaagttcgtgaccgccgccctgctgaataccccccctccttatcaggtgtcctgcggcggggaaagcgatagagccagcgcccgcgtcatcgaccctgccgcccagagcttcaccggagttgtgtacggaacccacacaaccgcagttagtgaaacaagacagacctgggccgagtgggcggctgcccattggtggcagctgaccctgggcgctatctgcgccctgctgctcgctggactgcttgcctgttgtgccaaatgcctgtactacctgcggggtgccatcgccccaagatgagctggagcctcggtggccatgcttcttgccccttgggcctccccccagcccctcctccccttcctgcacccgtacccccgtggtctttgaataaagtctgagtgggcggcaaaaaaaaaaaaaaaaaaaaaaaaaaaaaaagcatatgactaaaaaaaaaaaaaaaaaaaaaaaaaaaaaaaaaaaaaaaaaaaaaaaaaaaaaaaaaaaaaaaaaaaaaaaaaaagagacgccgctgatcagc

SEQ ID NO: 7 - DNA, 648 bp, unidentified
  source 1..648: mol_type = other DNA
atgtgtcaatcacgctacctcctctttttggccacccttgccctcctaaaccacctcagtttggccagggtcattccagtctctggacctgccaggtgtcttagccagtcccgaaacctgctgaagaccacagatgacatggtgaagacggccagagaaaaactgaaacattattcctgcactgctgaagacatcgatcatgaagacatcacacgggaccaaaccagcacattgaagacctgtttaccactggaactacacaagaacgagagttgcctggctactagagagacttcttccacaacaagagggagctgcctgcccccacagaagacgtctttgatgatgaccctgtgccttggtagcatctatgaggacttgaagatgtaccagacagagttccaggccatcaacgcagcacttcagaatcacaaccatcagcagatcattctagacaagggcatgctggtggccatcgatgagctgatgcagtctctgaatcataatggcgagactctgcgccagaaacctcctgtgggagaagcagacccttacagagtgaaaatgaagctctgcatcctgcttcacgccttcagcacccgcgtcgtgaccatcaacagggtgatgggctatctgagctccgcctga

SEQ ID NO: 8 - DNA, 1008 bp, unidentified
  source 1..1008: mol_type = other DNA
atgtgtcctcagaagctaaccatctcctggtttgccatcgttttgctggtgtctccactcatggccatgtgggagctggagaaagacgtttatgttgtagaggtggactggactcccgatgcccctggagaaacagtgaacctcacctgtgacacgcctgaagaagatgacatcacctggacctcagaccagagacatggagtcataggctctggaaagaccctgaccatcactgtcaaagagtttctagatgctggccagtacacctgccacaaaggaggcgagactctgagccactcacatctgctgctccacaagaaggaaaatggaatttggtccactgaaattttaaaaaatttcaaaaacaagactttcctgaagtgtgaagcaccaaattactccggacggttcacgtgctcatggctggtgcaaagaaacatggacttgaagttcaacatcaagagcagtagcagttcccctgactctcgggcagtgacatgtggaatggcgtctctgtctgcagagaaggtcacactggaccaaagggactatgagaagtattcagtgtcctgccaggaggatgtcacctgcccaactgccgaggagaccctgcccattgaactggcgttggaagcacggcagcagaataaatatgagaactacagcaccagcttcttcatcagggacatcatcaaaccagacccgcccaagaacttgcagatgaagcctttgaagaactcacaggtggaggtcagctgggagtaccctgactcctggagcactccccattcctacttctccctcaagttctttgttcgaatccagcgcaagaaagaaaagatgaaggagacagaggaggggtgtaaccagaaaggtgcgttcctcgtagagaagacatctaccgaagtccaatgcaaaggcgggaatgtctgcgtgcaagctcaggatcgctattacaattcctcatgcagcaagtgggcatgtgttccctgcagggtccgatcctag

SEQ ID NO: 9 - DNA, 2633 bp, synthetic construct
  source 1..2633: mol_type = other DNA
taatacgactcactataagagcagcgctgggtgttcaggggccaaggccaccatgtctggtcgtaaagctcagggaaaaaccctgggcgtcaatatggtacgacgaggagttcgctccttgtcaaacaaaataaaacaaaaaacaaaacaaattggaaacagacctggaccttcaagaggtgttcaaggatttatctttttctttttgttcaacattttgactggaaaaaagatcacagcccacctaaagaggttgtggaaaatgctggacccaagacaaggcttggctgttctaaggaaagtcaagagagtggtggccagtttgatgagaggattgtcctcaaggaaacgccgttcccatgatgttctgactgtgcaattcctaattttgggaatgctgttgatgacgggtggagtgaccttggtgcggaaaaacagatggttgctcctaaatgtgacatctgaggacctcgggaaaacattctctgtgggcacaggcaactgcacaacaaacattttggaagccaagtactggtgcccagactcaatggaatacaactgtcccaatctcagtccaagagaggagccagatgacattgattgctggtgctatggggtggaaaacgttagagtcgcatatggtaagtgtgactcagcaggcaggtctaggaggtcaagaagggccattgacttgcctacgcatgaaaaccatggtttgaagacccggcaagaaaaatggatgactggaagaatgggtgaaaggcaactccaaaagattgagagatggttcgtgaggaaccccttttttgcagtgacggctctgaccattgcctaccttgtgggaagcaacatgacgcaacgagtcgtgattgccctactggtcttggctgttggtccggcctactcagctcactgcattggaattactgacagggatttcattgagggggtgcatggaggaacttgggtttcagctaccctggagcaagacaagtgtgtcactgttatggcccctgacaagccttcattggacatctcactagagacagtagccattgatagacctgctgaggtgaggaaagtgtgttacaatgcagttctcactcatgtgaagattaatgacaagtgccccagcactggagaggcccacctagctgaagagaacgaaggggacaatgcgtgcaagcgcacttattctgatagaggctggggcaatggctgtggcctatttgggaaagggagcattgtggcatgcgccaaattcacttgtgccaaatccatgagtttgtttgaggttgatcagaccaaaattcagtatgtcatcagagcacaattgcatgtaggggccaagcaggaaaattggaataccgacattaagactctcaagtttgatgccctgtcaggctcccaggaagtcgagttcattgggtatggaaaagctacactggaatgccaggtgcaaactgcggtggactttggtaacagttacatcgctgagatggaaacagagagctggatagtggacagacagtgggcccaggacttgaccctgccatggcagagtggaagtggcggggtgtggagagagatgcatcatcttgtcgaatttgaacctccgcatgccgccactatcagagtactggccctgggaaaccaggaaggctccttgaaaacagctcttactggcgcaatgagggttacaaaggacacaaatgacaacaacctttacaaactacatggtggacatgtttcttgcagagtgaaattgtcagctttgacactcaaggggacatcctacaaaatatgcactgacaaaatgttttttgtcaagaacccaactgacactggccatggcactgttgtgatgcaggtgaaagtgtcaaaaggagccccctgcaggattccagtgatagtagctgatgatcttacagcggcaatcaataaaggcattttggttacagttaaccccatcgcctcaaccaatgatgatgaagtgctgattgaggtgaacccaccttttggagacagctacattatcgttgggagaggagattcacgtctcacttaccagtggcacaaagagggaagctcaataggaaagttgttcactcagaccatgaaaggcgtggaacgcctggccgtcatgggagacaccgcctgggatttcagctccgctggagggttcttcacttcggttgggaaaggaattcatacggtgtttggctctgcctttcaggggctatttggcggcttgaactggataacaaaggtcatcatgggggcggtacttatatgggttggcatcaacacaagaaacatgacaatgtccatgagcatgatcttggtaggagtgatcatgatgtttttgtctctaggagttggggcgtgagctggagcctcggtggccatgcttcttgccccttgggcctccccccagcccctcctccccttcctgcacccgtacccccgtggtctttgaataaagtctgagtgggcggcaaaaaaaaaaaaaaaaaaaaaaaaaaaaaaagcatatgactaaaaaaaaaaaaaaaaaaaaaaaaaaaaaaaaaaaaaaaaaaaaaaaaaaaaaaaaaaaaaaaaaaaaaaaaaaagagacgccgctgatcagc

SEQ ID NO: 10 - DNA, 2168 bp, synthetic construct
  source 1..2168: mol_type = other DNA
taatacgactcactataagagcagcgctgggtgttcaggggccaaggccaccatgggaaccgtgaacaagcctgtggtcggcgtgctgatgggctttggcattatcacaggcaccctgcggatcaccaaccctgtgcgggccagcgttctgagatacgacgacttccacatcgacgaggacaagctggacaccaacagcgtctacgagccctattaccattctgatcacgccgaatcttcttgggtgaatagaggcgagtctagcagaaaggcctatgaccacaactccccatacatttggcctcgtaacgactacgacggcttcctggaaaacgcccacgagcaccacggcgtgtacaaccagggaagaggcatcgacagcggagagagactgatgcagccaacccagatgagcgcccaggaggacctgggagacgacaccggcatccacgttatccccacactgaacggcgacgatagacacaagatcgtgaacgtggatcagagacagtacggcgatgtgttcaagggcgacctgaatcctaaacctcagggccaaagactgatcgaggtgtccgtggaagaaaatcaccccttcaccctgcgggcccctatccagcggatctacggcgtgcggtacacagagacatggtccttcctgccatctctgacctgcaccggggacgccgctcctgccatccaacacatctgtctgaagcacaccacctgcttccaggatgtggtcgtggacgtggattgcgccgaaaacacaaaagaagatcagctggccgagatcagctacagattccaagggaagaaggaggccgaccagccctggatcgtggtgaacaccagcacactgttcgacgagctggaactggaccctcctgagatcgagcctggcgtgctgaaagtgctgaggaccgagaaacagtacctgggcgtgtacatctggaatatgagaggcagcgacggcacctccacctacgccacatttctggtcacctggaagggcgatgagaagacccgcaaccccacccctgcagtgacccctcaacctagaggcgccgagttccacatgtggaactaccactctcatgtgttcagcgtgggcgacacgttctctctggctatgcacctgcagtataagatccacgaggctccttttgatctgctgctggaatggctgtacgtgcccatcgaccctacctgtcagcctatgcggctgtatagcacatgtctgtaccaccctaacgcccctcagtgcctgagccacatgaacagcggatgtacctttaccagcccgcacctggcccagagagtggccagcaccgtgtaccagaattgcgagcacgccgataactacaccgcctactgcctgggaattagccacatggaacccagctttggcctgatcctgcacgacggcggcacaacccttaaattcgtggacacacctgagagtctgagcggactgtacgtgttcgtggtgtacttcaacggccacgtggaagccgtggcctacaccgtggtctccaccgtggatcatttcgttaatgccatcgaggaacggggcttcccccccacagctggccagccacctgctacaacaaagcccaaggaaatcacacctgtgaaccccggcacaagcccactgctcagatacgccgcatggaccggcggcctggccgccgtggtgctgctatgcctggtgatcttcctgatctgcaccgccaagagaatgagagtgaaggcctaccgggtggacaaaagcccctacaaccagagcatgtactacgccggcctccctgttgacgacttcgaggacagcgagtccactgatacagaggaagaatttggcaacgccatcggcggtagccacggaggaagcagctacaccgtgtacatcgacaagaccagatgagctggagcctcggtggccatgcttcttgccccttgggcctccccccagcccctcctccccttcctgcacccgtacccccgtggtctttgaataaagtctgagtgggcggcaaaaaaaaaaaaaaaaaaaaaaaaaaaaaaagcatatgactaaaaaaaaaaaaaaaaaaaaaaaaaaaaaaaaaaaaaaaaaaaaaaaaaaaaaaaaaaaaaaaaaaaaaaaaaaagagacgccgctgatcagc

SEQ ID NO: 11 - DNA, 2657 bp, synthetic construct
  source 1..2657: mol_type = other DNA
taatacgactcactataagagcagcgctgggtgttcaggggccaaggccaccatgggcgctccccaggccttcctggccggcctgctgctggctgctgtggccgtgggcacagctagagccggcctccaacctagagccgacatggccgccccacccacactgcctcagccccctcgggcccacggccaacactacggccaccaccaccatcagctgccattcctgggccacgatggccaccacggcggcacactgagggtgggccagcaccacagaaacgccagcgacgtgctgcctgggcactggctgcagggaggctggggatgttacaacctgagcgactggcaccagggcacccacgtgtgccacaccaagcacatggacttctggtgcgtggaacacgacagaccccctcctgccacccccacaccactgacaaccgctgctaactctaccaccgccgccacacctgccaccgccccagctccatgtcacgccggcctgaacgacagctgtggcggctttctcagcggctgtggccctatgcggctgcggcacggcgctgacacccggtgcggcagactgatttgcggcctgtccaccacagcccaatacccccccaccagattcggctgcgccatgagatggggcctgcctccttgggagctggtggtgctgaccgcccggcctgaggacggctggacctgcagaggagtgccggcccacccaggcaccagatgtccagaactggtgtcccctatgggaagagccacctgttctcctgcttcagccctgtggctggctaccgccaacgccctgagcctggaccacgccctggccgcttttgtgctgctggtcccttgggtcctgatcttcatggtgtgcagaagaacatgtagaagacggggcgccgccgcggctctgacagccgtggtgctgcagggctacaaccccccagcctacggcgaggaagccttcacctacctctgcaccgcccctggctgcgccacccaagcccctgtgcctgtcagactggcaggcgtgcggtttgagagcaagatcgtggacggcggctgcttcgccccttgggacttggaggccaccggcgcctgcatctgcgaaatccctacagatgtgtcctgcgagggcctgggcgcttgggtgcccaccgcaccctgcgccagaatctggaacggaactcagcgagcctgcacattctgggctgtgaatgcctacagcagcggcggatacgcccagctggccagctacttcaaccctggcggttcttattacaagcagtaccaccctaccgcctgcgaggtggaacctgccttcggccattctgacgccgcctgctggggattccccacagatacagtgatgtctgtgttcgccctggccagctacgtgcagcacccacacaaaaccgtgagagttaagtttcacaccgagacaagaacagtctggcagctgagcgtggccggagtgtcttgtaacgtgacaacagagcatcccttctgcaacacccctcacggccagttagaggtgcaagtgcctcctgatcctggcgacctggtggagtacatcatgaaccacacaggcaaccagcagtccagatggggcctgggaagccccaactgccacggccctgattgggccagccctgtgtgtcagagacactctcctgactgcagccggctggtgggcgctacccctgaaagacctagactgcgcctggtggatgccgacgaccccctgctcagaaccgctcctggccccggcgaggtgtgggtcacacctgtgatcggcagccaggcccggaagtgcgggctgcacatcagagccggcccttacggccacgccaccgtcgaaatgcctgagtggattcacgcccacaccacaagcgacccctggcacccccccggccccctgggcttgaagttcaagaccgtgcggcccgtggccctgcctaggaccctggcccctcctcggaatgtgcgggtgaccggctgttaccagtgcggtactcccgctctggtggagggcctcgcccctggcggaggcaattgtcacctgaccgtcaacggagaggacctgggcgcctttcctcctggcaagttcgtgaccgccgccctgctgaataccccccctccttatcaggtgtcctgcggcggggaaagcgatagagccagcgcccgcgtcatcgaccctgccgcccagagcttcaccggagttgtgtacggaacccacacaaccgcagttagtgaaacaagacagacctgggccgagtgggcggctgcccattggtggcagctgaccctgggcgctatctgcgccctgctgctcgctggactgcttgcctgttgtgccaaatgcctgtactacctgcggggtgccatcgccccaagatgagctggagcctcggtggccatgcttcttgccccttgggcctccccccagcccctcctccccttcctgcacccgtacccccgtggtctttgaataaagtctgagtgggcggcaaaaaaaaaaaaaaaaaaaaaaaaaaaaaaagcatatgactaaaaaaaaaaaaaaaaaaaaaaaaaaaaaaaaaaaaaaaaaaaaaaaaaaaaaaaaaaaaaaaaaaaaaaaaaaagagacgccgctgatcagc

SEQ ID NO: 12 - protein, 778 aa, Yellow fever virus
MSGRKAQGKTLGVNMVRRGVRSLSNKIKQKTKQIGNRPGPSRGVQGFIFFFLFNILTGKKITAHLKRLWKMLDPRQGLAVLRKVKRVVASLMRGLSSRKRRSHDVLTVQFLILGMLLMTGGVTLVRKNRWLLLNVTSEDLGKTFSVGTGNCTTNILEAKYWCPDSMEYNCPNLSPREEPDDIDCWCYGVENVRVAYGKCDSAGRSRRSRRAIDLPTHENHGLKTRQEKWMTGRMGERQLQKIERWFVRNPFFAVTALTIAYLVGSNMTQRVVIALLVLAVGPAYSAHCIGITDRDFIEGVHGGTWVSATLEQDKCVTVMAPDKPSLDISLETVAIDRPAEVRKVCYNAVLTHVKINDKCPSTGEAHLAEENEGDNACKRTYSDRGWGNGCGLFGKGSIVACAKFTCAKSMSLFEVDQTKIQYVIRAQLHVGAKQENWNTDIKTLKFDALSGSQEVEFIGYGKATLECQVQTAVDFGNSYIAEMETESWIVDRQWAQDLTLPWQSGSGGVWREMHHLVEFEPPHAATIRVLALGNQEGSLKTALTGAMRVTKDTNDNNLYKLHGGHVSCRVKLSALTLKGTSYKICTDKMFFVKNPTDTGHGTVVMQVKVSKGAPCRIPVIVADDLTAAINKGILVTVNPIASTNDDEVLIEVNPPFGDSYIIVGRGDSRLTYQWHKEGSSIGKLFTQTMKGVERLAVMGDTAWDFSSAGGFFTSVGKGIHTVFGSAFQGLFGGLNWITKVIMGAVLIWVGINTRNMTMSMSMILVGVIMMFLSLGVGA

SEQ ID NO: 13 - protein, 623 aa, varicella-zoster virus
MGTVNKPVVGVLMGFGIITGTLRITNPVRASVLRYDDFHIDEDKLDTNSVYEPYYHSDHAESSWVNRGESSRKAYDHNSPYIWPRNDYDGFLENAHEHHGVYNQGRGIDSGERLMQPTQMSAQEDLGDDTGIHVIPTLNGDDRHKIVNVDQRQYGDVFKGDLNPKPQGQRLIEVSVEENHPFTLRAPIQRIYGVRYTETWSFLPSLTCTGDAAPAIQHICLKHTTCFQDVVVDVDCAENTKEDQLAEISYRFQGKKEADQPWIVVNTSTLFDELELDPPEIEPGVLKVLRTEKQYLGVYIWNMRGSDGTSTYATFLVTWKGDEKTRNPTPAVTPQPRGAEFHMWNYHSHVFSVGDTFSLAMHLQYKIHEAPFDLLLEWLYVPIDPTCQPMRLYSTCLYHPNAPQCLSHMNSGCTFTSPHLAQRVASTVYQNCEHADNYTAYCLGISHMEPSFGLILHDGGTTLKFVDTPESLSGLYVFVVYFNGHVEAVAYTVVSTVDHFVNAIEERGFPPTAGQPPATTKPKEITPVNPGTSPLLRYAAWTGGLAAVVLLCLVIFLICTAKRMRVKAYRVDKSPYNQSMYYAGLPVDDFEDSESTDTEEEFGNAIGGSHGGSSYTVYIDKTR

SEQ ID NO: 14 - protein, 786 aa, Rubella virus
MGAPQAFLAGLLLAAVAVGTARAGLQPRADMAAPPTLPQPPRAHGQHYGHHHHQLPFLGHDGHHGGTLRVGQHHRNASDVLPGHWLQGGWGCYNLSDWHQGTHVCHTKHMDFWCVEHDRPPPATPTPLTTAANSTTAATPATAPAPCHAGLNDSCGGFLSGCGPMRLRHGADTRCGRLICGLSTTAQYPPTRFGCAMRWGLPPWELVVLTARPEDGWTCRGVPAHPGTRCPELVSPMGRATCSPASALWLATANALSLDHALAAFVLLVPWVLIFMVCRRTCRRRGAAAALTAVVLQGYNPPAYGEEAFTYLCTAPGCATQAPVPVRLAGVRFESKIVDGGCFAPWDLEATGACICEIPTDVSCEGLGAWVPTAPCARIWNGTQRACTFWAVNAYSSGGYAQLASYFNPGGSYYKQYHPTACEVEPAFGHSDAACWGFPTDTVMSVFALASYVQHPHKTVRVKFHTETRTVWQLSVAGVSCNVTTEHPFCNTPHGQLEVQVPPDPGDLVEYIMNHTGNQQSRWGLGSPNCHGPDWASPVCQRHSPDCSRLVGATPERPRLRLVDADDPLLRTAPGPGEVWVTPVIGSQARKCGLHIRAGPYGHATVEMPEWIHAHTTSDPWHPPGPLGLKFKTVRPVALPRTLAPPRNVRVTGCYQCGTPALVEGLAPGGGNCHLTVNGEDLGAFPPGKFVTAALLNTPPPYQVSCGGESDRASARVIDPAAQSFTGVVYGTHTTAVSETRQTWAEWAAAHWWQLTLGAICALLLAGLLACCAKCLYYLRGAIAPR

SEQ ID NO: 15 - DNA, 1653 bp, unidentified
  source 1..1653: mol_type = genomic DNA
atggaagatgccaaaaacattaagaagggcccagcgccattctacccactcgaagacgggaccgccggcgagcagctgcacaaagccatgaagcgctacgccctggtgcccggcaccatcgcctttaccgacgcacatatcgaggtggacattacctacgccgagtacttcgagatgagcgttcggctggcagaagctatgaagcgctatgggctgaatacaaaccatcggatcgtggtgtgcagcgagaatagcttgcagttcttcatgcccgtgttgggtgccctgttcatcggtgtggctgtggccccagctaacgacatctacaacgagcgcgagctgctgaacagcatgggcatcagccagcccaccgtcgtattcgtgagcaagaaagggctgcaaaagatcctcaacgtgcaaaagaagctaccgatcatacaaaagatcatcatcatggatagcaagaccgactaccagggcttccaaagcatgtacaccttcgtgacttcccatttgccacccggcttcaacgagtacgacttcgtgcccgagagcttcgaccgggacaaaaccatcgccctgatcatgaacagtagtggcagtaccggattgcccaagggcgtagccctaccgcaccgcaccgcttgtgtccgattcagtcatgcccgcgaccccatcttcggcaaccagatcatccccgacaccgctatcctcagcgtggtgccatttcaccacggcttcggcatgttcaccacgctgggctacttgatctgcggctttcgggtcgtgctcatgtaccgcttcgaggaggagctattcttgcgcagcttgcaagactataagattcaatctgccctgctggtgcccacactatttagcttcttcgctaagagcactctcatcgacaagtacgacctaagcaacttgcacgagatcgccagcggcggggcgccgctcagcaaggaggtaggtgaggccgtggccaaacgcttccacctaccaggcatccgccagggctacggcctgacagaaacaaccagcgccattctgatcacccccgaaggggacgacaagcctggcgcagtaggcaaggtggtgcccttcttcgaggctaaggtggtggacttggacaccggtaagacactgggtgtgaaccagcgcggcgagctgtgcgtccgtggccccatgatcatgagcggctacgttaacaaccccgaggctacaaacgctctcatcgacaaggacggctggctgcacagcggcgacatcgcctactgggacgaggacgagcacttcttcatcgtggaccggctgaagagcctgatcaaatacaagggctaccaggtagccccagccgaactggagagcatcctgctgcaacaccccaacatcttcgacgccggggtcgccggcctgcccgacgacgatgccggcgagctgcccgccgcagtcgtcgtgctggaacacggtaaaaccatgaccgagaaggagatcgtggactatgtggccagccaggttacaaccgccaagaagctgcgcggtggtgttgtgttcgtggacgaggtgcctaaaggactgaccggcaagttggacgcccgcaagatccgcgagattctcattaaggccaagaagggcggcaagatcgccgtgtaa

SEQ ID NO: 16 - protein, 550 aa, unidentified
MEDAKNIKKGPAPFYPLEDGTAGEQLHKAMKRYALVPGTIAFTDAHIEVDITYAEYFEMSVRLAEAMKRYGLNTNHRIVVCSENSLQFFMPVLGALFIGVAVAPANDIYNERELLNSMGISQPTVVFVSKKGLQKILNVQKKLPIIQKIIIMDSKTDYQGFQSMYTFVTSHLPPGFNEYDFVPESFDRDKTIALIMNSSGSTGLPKGVALPHRTACVRFSHARDPIFGNQIIPDTAILSVVPFHHGFGMFTTLGYLICGFRVVLMYRFEEELFLRSLQDYKIQSALLVPTLFSFFAKSTLIDKYDLSNLHEIASGGAPLSKEVGEAVAKRFHLPGIRQGYGLTETTSAILITPEGDDKPGAVGKVVPFFEAKVVDLDTGKTLGVNQRGELCVRGPMIMSGYVNNPEATNALIDKDGWLHSGDIAYWDEDEHFFIVDRLKSLIKYKGYQVAPAELESILLQHPNIFDAGVAGLPDDDAGELPAAVVVLEHGKTMTEKEIVDYVASQVTTAKKLRGGVVFVDEVPKGLTGKLDARKIREILIKAKKGGKIAV

SEQ ID NO: 17 - DNA, 25 bp, synthetic construct
  source 1..25: mol_type = other DNA
taatacgactcactataagagcagc

SEQ ID NO: 18 - DNA, 18 bp, synthetic construct
  source 1..18: mol_type = other DNA
gctgatcagcggcgtctc

SEQ ID NO: 19 - DNA, 24 bp, synthetic construct
  source 1..24: mol_type = other DNA
atggaagatgccaaaaacattaag

SEQ ID NO: 20 - DNA, 19 bp, synthetic construct
  source 1..19: mol_type = other DNA
ttacacggcgatcttgccg

SEQ ID NO: 21 - DNA, 43 bp, synthetic construct
  source 1..43: mol_type = other DNA
taatacgactcactataagatggaagatgcctgaaaaacatta